European Patent Application EP 4 349 967 A1, published April 10, 2024. Title: NOVEL PLURIPOTENT CELL. Applicant: KOREA RESEARCH INSTITUTE OF BIOSCIENCE AND BIOTECHNOLOGY DAEGU GYEONGBUK INSTITUTE OF SCIENCE AND TECHNOLOGY. The sequence listing filed with the application follows.

SEQUENCE LISTING (98 sequences)

SEQ ID NO: 1 - DNA, 21 bp, Artificial Sequence
  nucleotide sequence for primer Nanog - forward primer
cctccagcagatgcaagaact

SEQ ID NO: 2 - DNA, 21 bp, Artificial Sequence
  nucleotide sequence for primer Nanog - reverse primer
cttcaaccactggtttttctg

SEQ ID NO: 3 - DNA, 21 bp, Artificial Sequence
  nucleotide sequence for primer Rex1 - forward primer
ggctgcgagaagagctttatt

SEQ ID NO: 4 - DNA, 20 bp, Artificial Sequence
  nucleotide sequence for primer Rex1 - reverse primer
agcatttcttcccggccttt

SEQ ID NO: 5 - DNA, 21 bp, Artificial Sequence
  nucleotide sequence for primer Esrrb - forward primer
aggctctcatttgggcctagc

SEQ ID NO: 6 - DNA, 20 bp, Artificial Sequence
  nucleotide sequence for primer Esrrb - reverse primer
atccttgcctgccacctgtt

SEQ ID NO: 7 - DNA, 20 bp, Artificial Sequence
  nucleotide sequence for primer Pax6 - forward primer
cgcggatctgtgttgctcat

SEQ ID NO: 8 - DNA, 21 bp, Artificial Sequence
  nucleotide sequence for primer Pax6 - reverse primer
cttaaatccatggcaaatctt

SEQ ID NO: 9 - DNA, 20 bp, Artificial Sequence
  nucleotide sequence for primer Sox1- forward primer
ggccgagtggaaggtcatgt

SEQ ID NO: 10 - DNA, 20 bp, Artificial Sequence
  nucleotide sequence for primer Sox1- reverse primer
tccgggtgttccttcatgtg

SEQ ID NO: 11 - DNA, 19 bp, Artificial Sequence
  nucleotide sequence for primer Map2- forward primer
gccagcctcggaacaaaca

SEQ ID NO: 12 - DNA, 20 bp, Artificial Sequence
  nucleotide sequence for primer Map2- reverse primer
gctcagcgaatgaggaagga

SEQ ID NO: 13 - DNA, 21 bp, Artificial Sequence
  nucleotide sequence for primer Dcx- forward primer
ccatgtgtgtgaggtgttgtg

SEQ ID NO: 14 - DNA, 21 bp, Artificial Sequence
  nucleotide sequence for primer Dcx- reverse primer
tcgatggagaacagagcttga

SEQ ID NO: 15 - DNA, 22 bp, Artificial Sequence
  nucleotide sequence for primer Dsp- forward primer
aatgaggagcttagcgaaatcc

SEQ ID NO: 16 - DNA, 22 bp, Artificial Sequence
  nucleotide sequence for primer Dsp- reverse primer
ccttcagttgcagataggtgag

SEQ ID NO: 17 - DNA, 21 bp, Artificial Sequence
  nucleotide sequence for primer Evpl- forward primer
aaccaggctttacaacaccag

SEQ ID NO: 18 - DNA, 21 bp, Artificial Sequence
  nucleotide sequence for primer Evpl- reverse primer
aggcggaagtaccatcttctc

SEQ ID NO: 19 - DNA, 22 bp, Artificial Sequence
  nucleotide sequence for primer Dsc1- forward primer
ggtcaaggaatcaaaacacagc

SEQ ID NO: 20 - DNA, 21 bp, Artificial Sequence
  nucleotide sequence for primer Dsc1- reverse primer
ccaagccgaggttgagtgaaa

SEQ ID NO: 21 - DNA, 20 bp, Artificial Sequence
  nucleotide sequence for primer Dsc2- forward primer
atggcggctgtgggatctat

SEQ ID NO: 22 - DNA, 20 bp, Artificial Sequence
  nucleotide sequence for primer Dsc2- reverse primer
gcaaggatcgcaagggtcaa

SEQ ID NO: 23 - DNA, 23 bp, Artificial Sequence
  nucleotide sequence for primer Dsc3- forward primer
agtttgaaagagtgtctcagctc

SEQ ID NO: 24 - DNA, 21 bp, Artificial Sequence
  nucleotide sequence for primer Dsc3- reverse primer
acaacagctctggtcggataa

SEQ ID NO: 25 - DNA, 20 bp, Artificial Sequence
  nucleotide sequence for primer Dsg1a- forward primer
actggctgggtaactggttc

SEQ ID NO: 26 - DNA, 21 bp, Artificial Sequence
  nucleotide sequence for primer Dsg1a- reverse primer
agggttagtgttagggcgagt

SEQ ID NO: 27 - DNA, 21 bp, Artificial Sequence
  nucleotide sequence for primer Dsg1b- forward primer
gcagtggtggtaatcgtgacc

SEQ ID NO: 28 - DNA, 21 bp, Artificial Sequence
  nucleotide sequence for primer Dsg1b- reverse primer
ggattttgcctaccgggagtg

SEQ ID NO: 29 - DNA, 22 bp, Artificial Sequence
  nucleotide sequence for primer Dsg1c- forward primer
catccactgagaaacctgtgac

SEQ ID NO: 30 - DNA, 19 bp, Artificial Sequence
  nucleotide sequence for primer Dsg1c- reverse primer
ctgtggcccttctacagcc

SEQ ID NO: 31 - DNA, 22 bp, Artificial Sequence
  nucleotide sequence for primer Dsg2- forward primer
cgtggttgaaggcattcatttc

SEQ ID NO: 32 - DNA, 21 bp, Artificial Sequence
  nucleotide sequence for primer Dsg2- reverse primer
tagctgcttgaccagtgtctt

SEQ ID NO: 33 - DNA, 19 bp, Artificial Sequence
  nucleotide sequence for primer Dsg3- forward primer
gccacggatgcagatgaac

SEQ ID NO: 34 - DNA, 19 bp, Artificial Sequence
  nucleotide sequence for primer Dsg3- reverse primer
cggacttctccggtgtttc

SEQ ID NO: 35 - DNA, 22 bp, Artificial Sequence
  nucleotide sequence for primer Dsg4- forward primer
ggtggtaaagttaagtgccaca

SEQ ID NO: 36 - DNA, 22 bp, Artificial Sequence
  nucleotide sequence for primer Dsg4- reverse primer
cttctccagtgtacctgttcac

SEQ ID NO: 37 - DNA, 20 bp, Artificial Sequence
  nucleotide sequence for primer Pkp1- forward primer
aaccactctccgctcaagac

SEQ ID NO: 38 - DNA, 21 bp, Artificial Sequence
  nucleotide sequence for primer Pkp1- reverse primer
cttctgccgtttgacggtcat

SEQ ID NO: 39 - DNA, 22 bp, Artificial Sequence
  nucleotide sequence for primer Jup- forward primer
tggcaacagacatacacctacg

SEQ ID NO: 40 - DNA, 22 bp, Artificial Sequence
  nucleotide sequence for primer Jup- reverse primer
ggtggtagtcttcttgagtgtg

SEQ ID NO: 41 - DNA, 21 bp, Artificial Sequence
  nucleotide sequence for primer Krt8- forward primer
tccatcagggtgactcagaaa

SEQ ID NO: 42 - DNA, 19 bp, Artificial Sequence
  nucleotide sequence for primer Krt8- reverse primer
ccagcttcaaggggctcaa

SEQ ID NO: 43 - DNA, 21 bp, Artificial Sequence
  nucleotide sequence for primer Krt16- forward primer
tggcgagaatatccactcctc

SEQ ID NO: 44 - DNA, 21 bp, Artificial Sequence
  nucleotide sequence for primer Krt16- reverse primer
tgaagctggttgaaccttgct

SEQ ID NO: 45 - DNA, 20 bp, Artificial Sequence
  nucleotide sequence for primer Krt17- forward primer
accatccgccagtttacctc

SEQ ID NO: 46 - DNA, 20 bp, Artificial Sequence
  nucleotide sequence for primer Krt17- reverse primer
actacccaggccactagctg

SEQ ID NO: 47 - DNA, 22 bp, Artificial Sequence
  nucleotide sequence for primer Shisa8- forward primer
ctctactcgtgctggtcggcat

SEQ ID NO: 48 - DNA, 23 bp, Artificial Sequence
  nucleotide sequence for primer Shisa8- reverse primer
acctggctgcttgagaagttctg

SEQ ID NO: 49 - DNA, 21 bp, Artificial Sequence
  nucleotide sequence for primer Cdk1- forward primer
agaaggtacttacggtgtggt

SEQ ID NO: 50 - DNA, 22 bp, Artificial Sequence
  nucleotide sequence for primer Cdk1- reverse primer
gagagatttcccgaattgcagt

SEQ ID NO: 51 - DNA, 20 bp, Artificial Sequence
  nucleotide sequence for primer Rpl7- forward primer
accgcactgagattcggatg

SEQ ID NO: 52 - DNA, 21 bp, Artificial Sequence
  nucleotide sequence for primer Rpl7- reverse primer
gaaccttacgaacctttgggc

SEQ ID NO: 53 - DNA, 21 bp, Artificial Sequence
  nucleotide sequence for primer Shisa3- forward primer
acctgtttgagacccaaggag

SEQ ID NO: 54 - DNA, 19 bp, Artificial Sequence
  nucleotide sequence for primer Shisa3- reverse primer
cagtggtgtaaggtggggg

SEQ ID NO: 55 - DNA, 19 bp, Artificial Sequence
  nucleotide sequence for primer Foxo4- forward primer
cttcctcgaccagacctcg

SEQ ID NO: 56 - DNA, 20 bp, Artificial Sequence
  nucleotide sequence for primer Foxo4- reverse primer
acaggatcggttcggagtgt

SEQ ID NO: 57 - DNA, 20 bp, Artificial Sequence
  nucleotide sequence for primer Ptp4a3- forward primer
catcactgttgtggactggc

SEQ ID NO: 58 - DNA, 20 bp, Artificial Sequence
  nucleotide sequence for primer Ptp4a3- reverse primer
tggatggcgtcctcgtactt

SEQ ID NO: 59 - DNA, 23 bp, Artificial Sequence
  nucleotide sequence for primer Blvra- forward primer
cctgattggatatgtgtccagac

SEQ ID NO: 60 - DNA, 20 bp, Artificial Sequence
  nucleotide sequence for primer Blvra- reverse primer
cgacatcaacctcttggctg

SEQ ID NO: 61 - DNA, 22 bp, Artificial Sequence
  nucleotide sequence for primer Mbnl3- forward primer
ttgattcactaaagggtcggtg

SEQ ID NO: 62 - DNA, 20 bp, Artificial Sequence
  nucleotide sequence for primer Mbnl3- reverse primer
ctgcggcagtcttctgttga

SEQ ID NO: 63 - DNA, 20 bp, Artificial Sequence
  nucleotide sequence for primer Mthfd2- forward primer
agtgcgaaatgaagccgttg

SEQ ID NO: 64 - DNA, 19 bp, Artificial Sequence
  nucleotide sequence for primer Mthfd2- reverse primer
gactggcgggattgtcacc

SEQ ID NO: 65 - DNA, 19 bp, Artificial Sequence
  nucleotide sequence for primer Dctpp1- forward primer
cgcggtactgtgggacaag

SEQ ID NO: 66 - DNA, 22 bp, Artificial Sequence
  nucleotide sequence for primer Dctpp1- reverse primer
caggctctgtatcagacttcca

SEQ ID NO: 67 - DNA, 21 bp, Artificial Sequence
  nucleotide sequence for primer DSP- forward primer
gcaggatgtactattctcggc

SEQ ID NO: 68 - DNA, 21 bp, Artificial Sequence
  nucleotide sequence for primer DSP- reverse primer
cctggatggtgttctggttct

SEQ ID NO: 69 - DNA, 19 bp, Artificial Sequence
  nucleotide sequence for primer RPL7- forward primer
ccaaattggcgtttgtcag

SEQ ID NO: 70 - DNA, 20 bp, Artificial Sequence
  nucleotide sequence for primer RPL7- reverse primer
gcatgttcgaagccttgttg

SEQ ID NO: 71 - DNA, 20 bp, Artificial Sequence
  nucleotide sequence for primer dspa- forward primer
gacctgcttctgaggtggac

SEQ ID NO: 72 - DNA, 20 bp, Artificial Sequence
  nucleotide sequence for primer dspa- reverse primer
ctcctggcttctctggattg

SEQ ID NO: 73 - DNA, 20 bp, Artificial Sequence
  nucleotide sequence for primer dspb- forward primer
gtcagggctcagagctgttc

SEQ ID NO: 74 - DNA, 20 bp, Artificial Sequence
  nucleotide sequence for primer dspb- reverse primer
tgaagacgcggtttctttct

SEQ ID NO: 75 - DNA, 20 bp, Artificial Sequence
  nucleotide sequence for primer msx1b- forward primer
caccttacgcaagcacaaga

SEQ ID NO: 76 - DNA, 20 bp, Artificial Sequence
  nucleotide sequence for primer msx1b- reverse primer
gtgaggttgagggagttgga

SEQ ID NO: 77 - DNA, 20 bp, Artificial Sequence
  nucleotide sequence for primer fgf20a- forward primer
tctcagagcagaggcagtca

SEQ ID NO: 78 - DNA, 20 bp, Artificial Sequence
  nucleotide sequence for primer fgf20a- reverse primer
tctctcgaccttccaggcta

SEQ ID NO: 79 - DNA, 20 bp, Artificial Sequence
  nucleotide sequence for primer her6- forward primer
ggttaacaccgaggtcagga

SEQ ID NO: 80 - DNA, 20 bp, Artificial Sequence
  nucleotide sequence for primer her6- reverse primer
tgaaccatgggttgactgaa

SEQ ID NO: 81 - DNA, 20 bp, Artificial Sequence
  nucleotide sequence for primer hspd1- forward primer
gtgttgacctgctggctgat

SEQ ID NO: 82 - DNA, 20 bp, Artificial Sequence
  nucleotide sequence for primer hspd1- reverse primer
accagcttggctccgatatt

SEQ ID NO: 83 - DNA, 20 bp, Artificial Sequence
  nucleotide sequence for primer rpl13a- forward primer
tctggaggactgtaagaggt

SEQ ID NO: 84 - DNA, 20 bp, Artificial Sequence
  nucleotide sequence for primer rpl13a- reverse primer
agacgcacaatcttgagagc

SEQ ID NO: 85 - DNA, 21 bp, Artificial Sequence
  shRNA for Dsp gene
gcctacaagaaaggtctcatt

SEQ ID NO: 86 - DNA, 20 bp, Artificial Sequence
  nucleotide sequence for primer junbb-forward probe
tgggttacggtcacaacgac

SEQ ID NO: 87 - DNA, 20 bp, Artificial Sequence
  nucleotide sequence for primer junbb- reverse probe
cagtgtccgttctcttccgt

SEQ ID NO: 88 - DNA, 25 bp, Artificial Sequence
  nucleotide sequence for pou5f3 MO
cgctctctccgtcatctttccgcta

SEQ ID NO: 89 - DNA, 25 bp, Artificial Sequence
  nucleotide sequence for dspa MO
aaactaaaaccgaggctgaccttct

SEQ ID NO: 90 - DNA, 25 bp, Artificial Sequence
  nucleotide sequence for dspb MO
ctgactgtgtttcagactgacctgt

SEQ ID NO: 91 - DNA, 52 bp, Artificial Sequence
  dspa sgRNA-1
taatacgactcactataggggagcctggtctgagaacgttttagagctagaa

SEQ ID NO: 92 - DNA, 52 bp, Artificial Sequence
  dspa sgRNA-2
taatacgactcactatagggccagacctcaccgccgtgttttagagctagaa

SEQ ID NO: 93 - DNA, 52 bp, Artificial Sequence
  dspa sgRNA-3
taatacgactcactatagggtaaactgtagccgacgggttttagagctagaa

SEQ ID NO: 94 - DNA, 52 bp, Artificial Sequence
  dspb sgRNA-1
taatacgactcactatagggttcaagaggcacagtcagttttagagctagaa

SEQ ID NO: 95 - DNA, 52 bp, Artificial Sequence
  dspb sgRNA-2
taatacgactcactataggaagtgcatctccagactggttttagagctagaa

SEQ ID NO: 96 - DNA, 52 bp, Artificial Sequence
  dspb sgRNA-3
taatacgactcactataggtgctgtgctcctgcaaacgttttagagctagaa

SEQ ID NO: 97 - DNA, 52 bp, Artificial Sequence
  Scrambled sgRNA
taatacgactcactatagcaggcaaagaatccctgccgttttagagctagaa

SEQ ID NO: 98 - DNA, 80 bp, Artificial Sequence
  sgRNA tail
aaaagcaccgactcggtgccactttttcaagttgataacggactagccttattttaacttgctatttctagctctaaaac